European Patent Specification EP 3 965 804 B1, published April 2, 2025. Title: BETA-LACTAMASE COMPOSITIONS FOR TREATMENT OF GRAFT VERSUS HOST DISEASE. Applicant: Synthetic Biologics, Inc. Memorial Sloan Kettering Cancer Center. The sequence listing filed with the application follows.

SEQUENCE LISTING (6 sequences)

SEQ ID NO: 1 - protein, 264 aa, Artificial Sequence
  Synthetic polymer.
TEMKDDFAKLEEQFDAKLGIFALDTGTNRTVAYRPDERFAFASTIKALTVGVLLQQKSIEDLNQRITYTRDDLVNYNPITEKHVDTGMTLKELADASLRYSDNAAQNLILKQIGGPESLKKELRKIGDEVTNPERFEPELNEVNPGETQDTSTARALVTSLRAFALEDKLPSEKRELLIDWMKRNTTGDALIRAGVPDGWEVADKTGAASYGTRNDIAIIWPPKGDPVVLAVLSSRDKKDAKYDNKLIAEATKVVMKALNMNGK

SEQ ID NO: 2 - DNA, 795 bp, Artificial Sequence
  Synthetic polymer.
atgactgagatgaaagatgattttgcgaagctggaagaacagtttgacgcaaaattgggcattttcgcgttggacacgggtacgaatcgtacggttgcctaccgtccggacgagcgcttcgccttcgcgagcacgatcaaagccctgaccgtcggcgtgctgctccagcaaaagagcatcgaggacctgaaccagcgcattacctacacccgtgatgatctggtgaactataatccgatcaccgagaaacacgttgataccggtatgaccctgaaagaactggcagatgcaagcctgcgctacagcgataacgcggctcagaatctgattctgaagcaaatcggtggtccggagagcttgaagaaagaactgcgtaaaatcggcgatgaagtcactaatccggagcgttttgagccggagctgaacgaagtgaatccgggtgaaacgcaagacacgagcaccgcgcgtgcgcttgtcacctccctgcgcgctttcgcactggaagataagctgccgtcggagaaacgcgagctgctgatcgactggatgaagcgcaatacgaccggcgacgcgctgattcgtgcgggcgttccggacggttgggaagtggctgacaagaccggtgcggcgagctacggcacccgtaacgatatcgcgatcatttggccacctaaaggtgacccggtcgtgctggccgtactgagcagccgtgacaagaaagacgcaaagtatgataacaagctgattgcagaggcgaccaaagttgttatgaaggcactgaacatgaatggtaag

SEQ ID NO: 3 - protein, 262 aa, Artificial Sequence
  Synthetic polymer.
EMKDDFAKLEEQFDAKLGIFALDTGTNRTVAYRPDERFAFASTIKALTVGVLLQQKSIEDLNQRITTRDDLVNYNPITEKHVDTGMTLKELADASLRYSDNAAQNLILKQIGGPESLKKELRKIGDEVTNPERFEPELNEVNPGETQDTSTARALVTSLRAFALEDKLPSEKRELLIDWMKRNTTGDALIRAGVPDGWEVGDKTGSGDYGTRNDIAIIWPPKGDPVVLAVLSSRDKKDAKYDNKLIAEATKVVMKALNMNGK

SEQ ID NO: 4 - protein, 299 aa, Artificial Sequence
  Synthetic polymer.
MIQKRKRTVSFRLVLMCTLLFVSLPITKTSAQASKTEMKDDFAKLEEQFDAKLGIFALDTGTNRTVAYRPDERFAFASTIKALTVGVLLQQKSIEDLNQRITYTRDDLVNYNPITEKHVDTGMTLKELADASLRYSDNAAQNLILKQIGGPESLKKELRKIGDEVTNPERFEPELNEVNPGETQDTSTARALVTSLRAFALEDKLPSEKRELLIDWMKRNTTGDALIRAGVPDGWEVGDKTGSGDYGTRNDIAIIWPPKGDPVVLAVLSSRDKKDAKYDNKLIAEATKVVMKALNMNGK

SEQ ID NO: 5 - DNA, 900 bp, Artificial Sequence
  Synthetic polymer.
atgattcaaaaacgaaagcggacagtttcgttcagacttgtgcttatgtgcacgctgttatttgtcagtttgccgattacaaaaacatcagcgcaagcttccaagacggagatgaaagatgattttgcaaaacttgaggaacaatttgatgcaaaactcgggatctttgcattggatacaggtacaaaccggacggtagcgtatcggccggatgagcgttttgcttttgcttcgacgattaaggctttaactgtaggcgtgcttttgcaacagaaatcaatagaagatctgaaccagagaataacatatacacgtgatgatcttgtaaactacaacccgattacggaaaagcacgttgatacgggaatgacgctcaaagagcttgcggatgcttcgcttcgatatagtgacaatgcggcacagaatctcattcttaaacaaattggcggacctgaaagtttgaaaaaggaactgaggaagattggtgatgaggttacaaatcccgaacgattcgaaccagagttaaatgaagtgaatccgggtgaaactcaggataccagtacagcaagagcacttgtcacaagccttcgagcctttgctcttgaagataaacttccaagtgaaaaacgcgagcttttaatcgattggatgaaacgaaataccactggagacgccttaatccgtgccggtgtgccggacggttgggaagtgggtgataaaactggaagcggagattatggaacccggaatgacattgccatcatttggccgccaaaaggagatcctgtcgttcttgcagtattatccagcagggataaaaaggacgccaagtatgataataaacttattgcagaggcaacaaaggtggtaatgaaagccttaaacatgaacggcaaataa

SEQ ID NO: 6 - protein, 216 aa, Artificial Sequence
  Synthetic polymer.
ETGTISISQLNKNVWVHTELGYFNGEAVPSNGLVLNTSKGLVLVDSSWDNKLTKELIEMVEKKFQKRVTDVIITHAHADRIGGITALKERGIKAHSTALTAELAKNSGYEEPLGDLQTITSLKFGNTKVETFYPGKGHTEDNIVVWLPQYQILAGGCLVKSAEAKDLGNVADAYVNEWSTSIENVLKRYGNINSVVPGHGEVGDKGLLLHTLDLLK